European Patent Application EP 4 397 771 A2, published July 10, 2024. Title: URINE STABILIZATION. Applicant: QIAGEN GmbH. Application EP. The sequence listing filed with the application follows.

SEQUENCE LISTING (9 sequences)

SEQ ID NO: 1 - DNA, 22 bp, synthetic construct
  misc_feature 1..22: note = Forw. Primer h 18S rDNA
  source 1..22: mol_type = other DNA
gccgctagaggtgaaattcttg

SEQ ID NO: 2 - DNA, 21 bp, synthetic construct
  misc_feature 1..21: note = h 18S rDNA Rev. Primer
  source 1..21: mol_type = other DNA
cattcttggcaaatgctttcg

SEQ ID NO: 3 - DNA, 21 bp, synthetic construct
  misc_feature 1..21: note = h 18S rDNA Probe
  source 1..21: mol_type = other DNA
accggcgcaagacggaccaga

SEQ ID NO: 4 - DNA, 22 bp, synthetic construct
  misc_feature 1..22: note = h18S rDNA 500bp amplicon Forward Primer
  source 1..22: mol_type = other DNA
gtcgctcgctcctctcctactt

SEQ ID NO: 5 - DNA, 19 bp, synthetic construct
  misc_feature 1..19: note = h18S rDNA 500bp amplicon Reverse Primer
  source 1..19: mol_type = other DNA
ggctgctggcaccagactt

SEQ ID NO: 6 - DNA, 25 bp, synthetic construct
  misc_feature 1..25: note = h18S rDNA 500bp amplicon Probe
  source 1..25: mol_type = other DNA
ctaatacatgccgacgggcgctgac

SEQ ID NO: 7 - DNA, 21 bp, synthetic construct
  misc_feature 1..21: note = DYS14 Forward Primer
  source 1..21: mol_type = other DNA
gagcaggcgtgggtactattg

SEQ ID NO: 8 - DNA, 19 bp, synthetic construct
  misc_feature 1..19: note = DYS14 Reverse Primer
  source 1..19: mol_type = other DNA
gtctgctgctcggcatcac

SEQ ID NO: 9 - DNA, 22 bp, synthetic construct
  misc_feature 1..22: note = DYS14 Probe
  source 1..22: mol_type = other DNA
cctgcatgcggcagagaaaccc